European Patent Application EP 4 722 238 A1, published April 8, 2026. Title: 一种基于胞内区截短体的嵌合抗原受体. Applicant: 中国科学院分子细胞科学卓越创新中心. The sequence listing filed with the application follows.

SEQUENCE LISTING (23 sequences)

SEQ ID NO: 1 - protein, 35 aa, synthetic construct
KNRKAKAKGGGGGGDYEPIRKGQRDLYSGLNQRRI

SEQ ID NO: 2 - protein, 41 aa, synthetic construct
RSKRSRLLHSDYMNMTPRRPGPTRKHYQPYAPPRDFAAYRS

SEQ ID NO: 3 - protein, 42 aa, synthetic construct
KRGRKKLLYIFKQPFMRPVQTTQEEDGCSCRFPEEEEGGCEL

SEQ ID NO: 4 - protein, 112 aa, synthetic construct
RVKFSRSADAPAYQQGQNQLYNELNLGRREEYDVLDKRRGRDPEMGGKPRRKNPQEGLYNELQKDKMAEAYSEIGMKGERRRGKGHDGLYQGLSTATKDTYDALHMQALPPR

SEQ ID NO: 5 - protein, 27 aa, synthetic construct
FWVLVVVGGVLACYSLLVTVAFIIFWV

SEQ ID NO: 6 - protein, 793 aa, synthetic construct
MVSKGEELFTGVVPILVELDGDVNGHKFSVSGEGEGDATYGKLTLKFICTTGKLPVPWPTLVTTLTYGVQCFSRYPDHMKQHDFFKSAMPEGYVQERTIFFKDDGNYKTRAEVKFEGDTLVNRIELKGIDFKEDGNILGHKLEYNYNSHNVYIMADKQKNGIKVNFKIRHNIEDGSVQLADHYQQNTPIGDGPVLLPDNHYLSTQSALSKDPNEKRDHMVLLEFVTAAGITLGMDELYKGSGEGRGSLLTCGDVEENPGPMLLLVTSLLLCELPHPAFLLIPYPYDVPDYADIQMTQTTSSLSASLGDRVTISCRASQDISKYLNWYQQKPDGTVKLLIYHTSRLHSGVPSRFSGSGSGTDYSLTISNLEQEDIATYFCQQGNTLPYTFGGGTKLEITGSTSGSGKPGSGEGSTKGEVKLQESGPGLVAPSQSLSVTCTVSGVSLPDYGVSWIRQPPRKGLEWLGVIWGSETTYYNSALKSRLTIIKDNSKSQVFLKMNSLQTDDTAIYYCAKHYYYGGSYAMDYWGQGTSVTVSSAAAIEVMYPPPYLDNEKSNGTIIHVKGKHLCPSPLFPGPSKPFWVLVVVGGVLACYSLLVTVAFIIFWVKNRKAKAKGGGGGGDYEPIRKGQRDLYSGLNQRRIRSKRSRLLHSDYMNMTPRRPGPTRKHYQPYAPPRDFAAYRSRVKFSRSADAPAYQQGQNQLYNELNLGRREEYDVLDKRRGRDPEMGGKPRRKNPQEGLYNELQKDKMAEAYSEIGMKGERRRGKGHDGLYQGLSTATKDTYDALHMQALPPR

SEQ ID NO: 7 - protein, 791 aa, synthetic construct
MVSKGEELFTGVVPILVELDGDVNGHKFSVSGEGEGDATYGKLTLKFICTTGKLPVPWPTLVTTLTYGVQCFSRYPDHMKQHDFFKSAMPEGYVQERTIFFKDDGNYKTRAEVKFEGDTLVNRIELKGIDFKEDGNILGHKLEYNYNSHNVYIMADKQKNGIKVNFKIRHNIEDGSVQLADHYQQNTPIGDGPVLLPDNHYLSTQSALSKDPNEKRDHMVLLEFVTAAGITLGMDELYKGSGEGRGSLLTCGDVEENPGPMLLLVTSLLLCELPHPAFLLIPYPYDVPDYADVVMTQSPLSLPVTPGEPASISCRSSQSLVHSNANTYLHWYLQKPGQSPQLLIYKVSNRFSGVPDRFSGSGSGTDFTLKISRVEAEDVGVYYCSQNTHVPPTFGQGTKLEIKRGGGGSGGGGSGGGGSQVQLVQSGAEVKKPGASVKVSCKASGYTFTDYEMHWVRQAPGQGLEWMGALDPKTGDTAYSQKFKGRVTLTADESTSTAYMELSSLRSEDTAVYYCTRFYSYTYWGQGTLVTVSSAAAIEVMYPPPYLDNEKSNGTIIHVKGKHLCPSPLFPGPSKPFWVLVVVGGVLACYSLLVTVAFIIFWVKNRKAKAKGGGGGGDYEPIRKGQRDLYSGLNQRRIRSKRSRLLHSDYMNMTPRRPGPTRKHYQPYAPPRDFAAYRSRVKFSRSADAPAYQQGQNQLYNELNLGRREEYDVLDKRRGRDPEMGGKPRRKNPQEGLYNELQKDKMAEAYSEIGMKGERRRGKGHDGLYQGLSTATKDTYDALHMQALPPR

SEQ ID NO: 8 - DNA, 2382 bp, synthetic construct
  source 1..2382: mol_type = other DNA
atggtgagcaagggcgaggagctgttcaccggggtggtgcccatcctggtcgagctggacggcgacgtaaacggccacaagttcagcgtgtccggcgagggcgagggcgatgccacctacggcaagctgaccctgaagttcatctgcaccaccggcaagctgcccgtgccctggcccaccctcgtgaccaccctgacctacggcgtgcagtgcttcagccgctaccccgaccacatgaagcagcacgacttcttcaagtccgccatgcccgaaggctacgtccaggagcgcaccatcttcttcaaggacgacggcaactacaagacccgcgccgaggtgaagttcgagggcgacaccctggtgaaccgcatcgagctgaagggcatcgacttcaaggaggacggcaacatcctggggcacaagctggagtacaactacaacagccacaacgtctatatcatggccgacaagcagaagaacggcatcaaggtgaacttcaagatccgccacaacatcgaggacggcagcgtgcagctcgccgaccactaccagcagaacacccccatcggcgacggccccgtgctgctgcccgacaaccactacctgagcacccagtccgccctgagcaaagaccccaacgagaagcgcgatcacatggtcctgctggagttcgtgaccgccgccgggatcactctcggcatggacgagctgtacaagggaagcggagagggcagaggaagtctgctaacatgcggtgacgtcgaggagaatcctggacctatgcttctcctggtgacaagccttctgctctgtgagttaccacacccagcattcctcctgatcccatacccctacgacgtgcccgactacgccgacatccagatgacacagactacatcctccctgtctgcctctctgggagacagagtcaccatcagttgcagggcaagtcaggacattagtaaatatttaaattggtatcagcagaaaccagatggaactgttaaactcctgatctaccatacatcaagattacactcaggagtcccatcaaggttcagtggcagtgggtctggaacagattattctctcaccattagcaacctggagcaagaagatattgccacttacttttgccaacagggtaatacgcttccgtacacgttcggaggggggactaagttggaaataacaggctccacctctggatccggcaagcccggatctggcgagggatccaccaagggcgaggtgaaactgcaggagtcaggacctggcctggtggcgccctcacagagcctgtccgtcacatgcactgtctcaggggtctcattacccgactatggtgtaagctggattcgccagcctccacgaaagggtctggagtggctgggagtaatatggggtagtgaaaccacatactataattcagctctcaaatccagactgaccatcatcaaggacaactccaagagccaagttttcttaaaaatgaacagtctgcaaactgatgacacagccatttactactgtgccaaacattattactacggtggtagctatgctatggactactggggtcaaggaacctcagtcaccgtctcctcagcggccgcaattgaagttatgtatcctcctccttacctagacaatgagaagagcaatggaaccattatccatgtgaaagggaaacacctttgtccaagtcccctatttcccggaccttctaagcccttttgggtgctggtggtggttgggggagtcctggcttgctatagcttgctagtaacagtggcctttattattttctgggtgaagaatagaaaagccaaggctaaaggcggagggggtggcggagactatgagcccatccggaaaggccagcgggacctgtattctggcctgaatcagagacgcatcaggagtaagaggagcaggctcctgcacagtgactacatgaacatgactccccgccgccccgggcccacccgcaagcattaccagccctatgccccaccacgcgacttcgcagcctatcgctccagagtgaagttcagcaggagcgcagacgcccccgcgtaccagcagggccagaaccagctctataacgagctcaatctaggacgaagagaggagtacgatgttttggacaagagacgtggccgggaccctgagatggggggaaagccgagaaggaagaaccctcaggaaggcctgtacaatgaactgcagaaagataagatggcggaggcctacagtgagattgggatgaaaggcgagcgccggaggggcaaggggcacgatggcctttaccagggtctcagtacagccaccaaggacacctacgacgcccttcacatgcaggccctgccccctcgctaa

SEQ ID NO: 9 - DNA, 2376 bp, synthetic construct
  source 1..2376: mol_type = other DNA
atggtgagcaagggcgaggagctgttcaccggggtggtgcccatcctggtcgagctggacggcgacgtaaacggccacaagttcagcgtgtccggcgagggcgagggcgatgccacctacggcaagctgaccctgaagttcatctgcaccaccggcaagctgcccgtgccctggcccaccctcgtgaccaccctgacctacggcgtgcagtgcttcagccgctaccccgaccacatgaagcagcacgacttcttcaagtccgccatgcccgaaggctacgtccaggagcgcaccatcttcttcaaggacgacggcaactacaagacccgcgccgaggtgaagttcgagggcgacaccctggtgaaccgcatcgagctgaagggcatcgacttcaaggaggacggcaacatcctggggcacaagctggagtacaactacaacagccacaacgtctatatcatggccgacaagcagaagaacggcatcaaggtgaacttcaagatccgccacaacatcgaggacggcagcgtgcagctcgccgaccactaccagcagaacacccccatcggcgacggccccgtgctgctgcccgacaaccactacctgagcacccagtccgccctgagcaaagaccccaacgagaagcgcgatcacatggtcctgctggagttcgtgaccgccgccgggatcactctcggcatggacgagctgtacaagggaagcggagagggcagaggaagtctgctaacatgcggtgacgtcgaggagaatcctggacctatgcttctcctggtgacaagccttctgctctgtgagttaccacacccagcattcctcctgatcccatacccctacgacgtgcccgactacgccgatgttgtgatgactcagtctccactctccctgcccgtcacccctggagagccggcctccatctcctgcagatctagtcagagccttgtacacagtaatgccaacacctatttacattggtacctgcagaagccagggcagtctccacagctcctgatctataaagtttccaaccgattttctggggtccctgacaggttcagtggcagtggatcaggcacagattttacactgaaaatcagcagagtggaggctgaggatgttggggtttattactgctctcaaaatacacatgttcctcctacgtttggccaggggaccaagctggagatcaaacgtggtggaggcggttcaggcggaggtggctctggcggtggcggatcgcaggtgcagctggtgcagtctggagctgaggtgaagaagcctggggcctcagtgaaggtctcctgcaaggcttctggatacaccttcaccgactatgaaatgcactgggtgcgacaggcccctggacaagggcttgagtggatgggagctcttgatcctaaaactggtgatactgcctacagtcagaagttcaagggcagagtcacgctgaccgcggacgaatccacgagcacagcctacatggagctgagcagcctgagatctgaggacacggccgtgtattactgtacaagattctactcctatacttactggggccagggaaccctggtcaccgtctcctcagcggccgcaattgaagttatgtatcctcctccttacctagacaatgagaagagcaatggaaccattatccatgtgaaagggaaacacctttgtccaagtcccctatttcccggaccttctaagcccttttgggtgctggtggtggttgggggagtcctggcttgctatagcttgctagtaacagtggcctttattattttctgggtgaagaatagaaaagccaaggctaaaggcggagggggtggcggagactatgagcccatccggaaaggccagcgggacctgtattctggcctgaatcagagacgcatcaggagtaagaggagcaggctcctgcacagtgactacatgaacatgactccccgccgccccgggcccacccgcaagcattaccagccctatgccccaccacgcgacttcgcagcctatcgctccagagtgaagttcagcaggagcgcagacgcccccgcgtaccagcagggccagaaccagctctataacgagctcaatctaggacgaagagaggagtacgatgttttggacaagagacgtggccgggaccctgagatggggggaaagccgagaaggaagaaccctcaggaaggcctgtacaatgaactgcagaaagataagatggcggaggcctacagtgagattgggatgaaaggcgagcgccggaggggcaaggggcacgatggcctttaccagggtctcagtacagccaccaaggacacctacgacgcccttcacatgcaggccctgccccctcgctaa

SEQ ID NO: 10 - protein, 245 aa, synthetic construct
DIQMTQTTSSLSASLGDRVTISCRASQDISKYLNWYQQKPDGTVKLLIYHTSRLHSGVPSRFSGSGSGTDYSLTISNLEQEDIATYFCQQGNTLPYTFGGGTKLEITGSTSGSGKPGSGEGSTKGEVKLQESGPGLVAPSQSLSVTCTVSGVSLPDYGVSWIRQPPRKGLEWLGVIWGSETTYYNSALKSRLTIIKDNSKSQVFLKMNSLQTDDTAIYYCAKHYYYGGSYAMDYWGQGTSVTVSS

SEQ ID NO: 11 - protein, 243 aa, synthetic construct
DVVMTQSPLSLPVTPGEPASISCRSSQSLVHSNANTYLHWYLQKPGQSPQLLIYKVSNRFSGVPDRFSGSGSGTDFTLKISRVEAEDVGVYYCSQNTHVPPTFGQGTKLEIKRGGGGSGGGGSGGGGSQVQLVQSGAEVKKPGASVKVSCKASGYTFTDYEMHWVRQAPGQGLEWMGALDPKTGDTAYSQKFKGRVTLTADESTSTAYMELSSLRSEDTAVYYCTRFYSYTYWGQGTLVTVSS

SEQ ID NO: 12 - DNA, 2349 bp, synthetic construct
  source 1..2349: mol_type = other DNA
atggtgagcaagggcgaggagctgttcaccggggtggtgcccatcctggtcgagctggacggcgacgtaaacggccacaagttcagcgtgtccggcgagggcgagggcgatgccacctacggcaagctgaccctgaagttcatctgcaccaccggcaagctgcccgtgccctggcccaccctcgtgaccaccctgacctacggcgtgcagtgcttcagccgctaccccgaccacatgaagcagcacgacttcttcaagtccgccatgcccgaaggctacgtccaggagcgcaccatcttcttcaaggacgacggcaactacaagacccgcgccgaggtgaagttcgagggcgacaccctggtgaaccgcatcgagctgaagggcatcgacttcaaggaggacggcaacatcctggggcacaagctggagtacaactacaacagccacaacgtctatatcatggccgacaagcagaagaacggcatcaaggtgaacttcaagatccgccacaacatcgaggacggcagcgtgcagctcgccgaccactaccagcagaacacccccatcggcgacggccccgtgctgctgcccgacaaccactacctgagcacccagtccgccctgagcaaagaccccaacgagaagcgcgatcacatggtcctgctggagttcgtgaccgccgccgggatcactctcggcatggacgagctgtacaagggaagcggagagggcagaggaagtctgctaacatgcggtgacgtcgaggagaatcctggacctatgcttctcctggtgacaagccttctgctctgtgagttaccacacccagcattcctcctgatcccatacccctacgacgtgcccgactacgcccaggtacaactgcagcagtctgggcctgagctggagaagcctggcgcttcagtgaagatatcctgcaaggcttctggttactcattcactggctacaccatgaactgggtgaagcagagccatggaaagagccttgagtggattggacttattactccttacaatggtgcttctagctacaaccagaagttcaggggcaaggccacattaactgtagacaagtcatccagcacagcctacatggacctcctcagtctgacatctgaagactctgcagtctatttctgtgcaagggggggttacgacgggaggggttttgactactggggccaagggaccacggtcaccgtctcctcaggtggaggcggttcaggcggcggtggctctagcggtggtggatcggacatcgagctcactcagtctccagcaatcatgtctgcatctccaggggagaaggtcaccatgacctgcagtgccagctcaagtgtaagttacatgcactggtaccagcagaagtcaggcacctcccccaaaagatggatttatgacacatccaaactggcttctggagtcccaggtcgcttcagtggcagtgggtctggaaactcttactctctcacaatcagcagcgtggaggctgaagatgatgcaacttattactgccagcagtggagtaagcaccctctcacgtacggtgctgggacaaagttggaaatcaaagcggccgcaattgaagttatgtatcctcctccttacctagacaatgagaagagcaatggaaccattatccatgtgaaagggaaacacctttgtccaagtcccctatttcccggaccttctaagcccttttgggtgctggtggtggttgggggagtcctggcttgctatagcttgctagtaacagtggcctttattattttctgggtgaagaatagaaaggccaaggccaaggactatgagcccatccggaaaggccagcgggacctgtattctggcctgaatcagagacgcatcaggagtaagaggagcaggctcctgcacagtgactacatgaacatgactccccgccgccccgggcccacccgcaagcattaccagccctatgccccaccacgcgacttcgcagcctatcgctccagagtgaagttcagcaggagcgcagacgcccccgcgtaccagcagggccagaaccagctctataacgagctcaatctaggacgaagagaggagtacgatgttttggacaagagacgtggccgggaccctgagatggggggaaagccgagaaggaagaaccctcaggaaggcctgtacaatgaactgcagaaagataagatggcggaggcctacagtgagattgggatgaaaggcgagcgccggaggggcaaggggcacgatggcctttaccagggtctcagtacagccaccaaggacacctacgacgcccttcacatgcaggccctgccccctcgctaa

SEQ ID NO: 13 - DNA, 2358 bp, synthetic construct
  source 1..2358: mol_type = other DNA
atggtgagcaagggcgaggagctgttcaccggggtggtgcccatcctggtcgagctggacggcgacgtaaacggccacaagttcagcgtgtccggcgagggcgagggcgatgccacctacggcaagctgaccctgaagttcatctgcaccaccggcaagctgcccgtgccctggcccaccctcgtgaccaccctgacctacggcgtgcagtgcttcagccgctaccccgaccacatgaagcagcacgacttcttcaagtccgccatgcccgaaggctacgtccaggagcgcaccatcttcttcaaggacgacggcaactacaagacccgcgccgaggtgaagttcgagggcgacaccctggtgaaccgcatcgagctgaagggcatcgacttcaaggaggacggcaacatcctggggcacaagctggagtacaactacaacagccacaacgtctatatcatggccgacaagcagaagaacggcatcaaggtgaacttcaagatccgccacaacatcgaggacggcagcgtgcagctcgccgaccactaccagcagaacacccccatcggcgacggccccgtgctgctgcccgacaaccactacctgagcacccagtccgccctgagcaaagaccccaacgagaagcgcgatcacatggtcctgctggagttcgtgaccgccgccgggatcactctcggcatggacgagctgtacaagggaagcggagagggcagaggaagtctgctaacatgcggtgacgtcgaggagaatcctggacctatgcttctcctggtgacaagccttctgctctgtgagttaccacacccagcattcctcctgatcccatacccctacgacgtgcccgactacgcccaggtacaactgcagcagtctgggcctgagctggagaagcctggcgcttcagtgaagatatcctgcaaggcttctggttactcattcactggctacaccatgaactgggtgaagcagagccatggaaagagccttgagtggattggacttattactccttacaatggtgcttctagctacaaccagaagttcaggggcaaggccacattaactgtagacaagtcatccagcacagcctacatggacctcctcagtctgacatctgaagactctgcagtctatttctgtgcaagggggggttacgacgggaggggttttgactactggggccaagggaccacggtcaccgtctcctcaggtggaggcggttcaggcggcggtggctctagcggtggtggatcggacatcgagctcactcagtctccagcaatcatgtctgcatctccaggggagaaggtcaccatgacctgcagtgccagctcaagtgtaagttacatgcactggtaccagcagaagtcaggcacctcccccaaaagatggatttatgacacatccaaactggcttctggagtcccaggtcgcttcagtggcagtgggtctggaaactcttactctctcacaatcagcagcgtggaggctgaagatgatgcaacttattactgccagcagtggagtaagcaccctctcacgtacggtgctgggacaaagttggaaatcaaagcggccgcaattgaagttatgtatcctcctccttacctagacaatgagaagagcaatggaaccattatccatgtgaaagggaaacacctttgtccaagtcccctatttcccggaccttctaagcccttttgggtgctggtggtggttgggggagtcctggcttgctatagcttgctagtaacagtggcctttattattttctgggtgaagaatagaaaagccaaggctaagggcggaggagactatgagcccatccggaaaggccagcgggacctgtattctggcctgaatcagagacgcatcaggagtaagaggagcaggctcctgcacagtgactacatgaacatgactccccgccgccccgggcccacccgcaagcattaccagccctatgccccaccacgcgacttcgcagcctatcgctccagagtgaagttcagcaggagcgcagacgcccccgcgtaccagcagggccagaaccagctctataacgagctcaatctaggacgaagagaggagtacgatgttttggacaagagacgtggccgggaccctgagatggggggaaagccgagaaggaagaaccctcaggaaggcctgtacaatgaactgcagaaagataagatggcggaggcctacagtgagattgggatgaaaggcgagcgccggaggggcaaggggcacgatggcctttaccagggtctcagtacagccaccaaggacacctacgacgcccttcacatgcaggccctgccccctcgctaa

SEQ ID NO: 14 - protein, 33 aa, synthetic construct
KNRKAKAKGGGGDYEPIRKGQRDLYSGLNQRRI

SEQ ID NO: 15 - protein, 34 aa, synthetic construct
KNRKAKAKGGGGGDYEPIRKGQRDLYSGLNQRRI

SEQ ID NO: 16 - protein, 36 aa, synthetic construct
KNRKAKAKGGGGGGGDYEPIRKGQRDLYSGLNQRRI

SEQ ID NO: 17 - protein, 37 aa, synthetic construct
KNRKAKAKGGGGGGGGDYEPIRKGQRDLYSGLNQRRI

SEQ ID NO: 18 - DNA, 2376 bp, synthetic construct
  source 1..2376: mol_type = other DNA
atggtgagcaagggcgaggagctgttcaccggggtggtgcccatcctggtcgagctggacggcgacgtaaacggccacaagttcagcgtgtccggcgagggcgagggcgatgccacctacggcaagctgaccctgaagttcatctgcaccaccggcaagctgcccgtgccctggcccaccctcgtgaccaccctgacctacggcgtgcagtgcttcagccgctaccccgaccacatgaagcagcacgacttcttcaagtccgccatgcccgaaggctacgtccaggagcgcaccatcttcttcaaggacgacggcaactacaagacccgcgccgaggtgaagttcgagggcgacaccctggtgaaccgcatcgagctgaagggcatcgacttcaaggaggacggcaacatcctggggcacaagctggagtacaactacaacagccacaacgtctatatcatggccgacaagcagaagaacggcatcaaggtgaacttcaagatccgccacaacatcgaggacggcagcgtgcagctcgccgaccactaccagcagaacacccccatcggcgacggccccgtgctgctgcccgacaaccactacctgagcacccagtccgccctgagcaaagaccccaacgagaagcgcgatcacatggtcctgctggagttcgtgaccgccgccgggatcactctcggcatggacgagctgtacaagggaagcggagagggcagaggaagtctgctaacatgcggtgacgtcgaggagaatcctggacctatgcttctcctggtgacaagccttctgctctgtgagttaccacacccagcattcctcctgatcccatacccctacgacgtgcccgactacgcccaggtacaactgcagcagtctgggcctgagctggagaagcctggcgcttcagtgaagatatcctgcaaggcttctggttactcattcactggctacaccatgaactgggtgaagcagagccatggaaagagccttgagtggattggacttattactccttacaatggtgcttctagctacaaccagaagttcaggggcaaggccacattaactgtagacaagtcatccagcacagcctacatggacctcctcagtctgacatctgaagactctgcagtctatttctgtgcaagggggggttacgacgggaggggttttgactactggggccaagggaccacggtcaccgtctcctcaggtggaggcggttcaggcggcggtggctctagcggtggtggatcggacatcgagctcactcagtctccagcaatcatgtctgcatctccaggggagaaggtcaccatgacctgcagtgccagctcaagtgtaagttacatgcactggtaccagcagaagtcaggcacctcccccaaaagatggatttatgacacatccaaactggcttctggagtcccaggtcgcttcagtggcagtgggtctggaaactcttactctctcacaatcagcagcgtggaggctgaagatgatgcaacttattactgccagcagtggagtaagcaccctctcacgtacggtgctgggacaaagttggaaatcaaagcggccgcaattgaagttatgtatcctcctccttacctagacaatgagaagagcaatggaaccattatccatgtgaaagggaaacacctttgtccaagtcccctatttcccggaccttctaagcccttttgggtgctggtggtggttgggggagtcctggcttgctatagcttgctagtaacagtggcctttattattttctgggtgaagaatagaaaagccaaggctaaaggcggaggtggtggcggaggaggtggagactatgagcccatccggaaaggccagcgggacctgtattctggcctgaatcagagacgcatcaggagtaagaggagcaggctcctgcacagtgactacatgaacatgactccccgccgccccgggcccacccgcaagcattaccagccctatgccccaccacgcgacttcgcagcctatcgctccagagtgaagttcagcaggagcgcagacgcccccgcgtaccagcagggccagaaccagctctataacgagctcaatctaggacgaagagaggagtacgatgttttggacaagagacgtggccgggaccctgagatggggggaaagccgagaaggaagaaccctcaggaaggcctgtacaatgaactgcagaaagataagatggcggaggcctacagtgagattgggatgaaaggcgagcgccggaggggcaaggggcacgatggcctttaccagggtctcagtacagccaccaaggacacctacgacgcccttcacatgcaggccctgccccctcgctaa

SEQ ID NO: 19 - DNA, 2364 bp, synthetic construct
  source 1..2364: mol_type = other DNA
atggtgagcaagggcgaggagctgttcaccggggtggtgcccatcctggtcgagctggacggcgacgtaaacggccacaagttcagcgtgtccggcgagggcgagggcgatgccacctacggcaagctgaccctgaagttcatctgcaccaccggcaagctgcccgtgccctggcccaccctcgtgaccaccctgacctacggcgtgcagtgcttcagccgctaccccgaccacatgaagcagcacgacttcttcaagtccgccatgcccgaaggctacgtccaggagcgcaccatcttcttcaaggacgacggcaactacaagacccgcgccgaggtgaagttcgagggcgacaccctggtgaaccgcatcgagctgaagggcatcgacttcaaggaggacggcaacatcctggggcacaagctggagtacaactacaacagccacaacgtctatatcatggccgacaagcagaagaacggcatcaaggtgaacttcaagatccgccacaacatcgaggacggcagcgtgcagctcgccgaccactaccagcagaacacccccatcggcgacggccccgtgctgctgcccgacaaccactacctgagcacccagtccgccctgagcaaagaccccaacgagaagcgcgatcacatggtcctgctggagttcgtgaccgccgccgggatcactctcggcatggacgagctgtacaagggaagcggagagggcagaggaagtctgctaacatgcggtgacgtcgaggagaatcctggacctatgcttctcctggtgacaagccttctgctctgtgagttaccacacccagcattcctcctgatcccatacccctacgacgtgcccgactacgcccaggtacaactgcagcagtctgggcctgagctggagaagcctggcgcttcagtgaagatatcctgcaaggcttctggttactcattcactggctacaccatgaactgggtgaagcagagccatggaaagagccttgagtggattggacttattactccttacaatggtgcttctagctacaaccagaagttcaggggcaaggccacattaactgtagacaagtcatccagcacagcctacatggacctcctcagtctgacatctgaagactctgcagtctatttctgtgcaagggggggttacgacgggaggggttttgactactggggccaagggaccacggtcaccgtctcctcaggtggaggcggttcaggcggcggtggctctagcggtggtggatcggacatcgagctcactcagtctccagcaatcatgtctgcatctccaggggagaaggtcaccatgacctgcagtgccagctcaagtgtaagttacatgcactggtaccagcagaagtcaggcacctcccccaaaagatggatttatgacacatccaaactggcttctggagtcccaggtcgcttcagtggcagtgggtctggaaactcttactctctcacaatcagcagcgtggaggctgaagatgatgcaacttattactgccagcagtggagtaagcaccctctcacgtacggtgctgggacaaagttggaaatcaaagcggccgcaattgaagttatgtatcctcctccttacctagacaatgagaagagcaatggaaccattatccatgtgaaagggaaacacctttgtccaagtcccctatttcccggaccttctaagcccttttgggtgctggtggtggttgggggagtcctggcttgctatagcttgctagtaacagtggcctttattattttctgggtgaagaatagaaaagccaaggctaaaggcggagggggtggcggagactatgagcccatccggaaaggccagcgggacctgtattctggcctgaatcagagacgcatcaggagtaagaggagcaggctcctgcacagtgactacatgaacatgactccccgccgccccgggcccacccgcaagcattaccagccctatgccccaccacgcgacttcgcagcctatcgctccagagtgaagttcagcaggagcgcagacgcccccgcgtaccagcagggccagaaccagctctataacgagctcaatctaggacgaagagaggagtacgatgttttggacaagagacgtggccgggaccctgagatggggggaaagccgagaaggaagaaccctcaggaaggcctgtacaatgaactgcagaaagataagatggcggaggcctacagtgagattgggatgaaaggcgagcgccggaggggcaaggggcacgatggcctttaccagggtctcagtacagccaccaaggacacctacgacgcccttcacatgcaggccctgccccctcgc

SEQ ID NO: 20 - protein, 240 aa, synthetic construct
QVQLQQSGPELEKPGASVKISCKASGYSFTGYTMNWVKQSHGKSLEWIGLITPYNGASSYNQKFRGKATLTVDKSSSTAYMDLLSLTSEDSAVYFCARGGYDGRGFDYWGQGTTVTVSSGGGGSGGGGSSGGGSDIELTQSPAIMSASPGEKVTMTCSASSSVSYMHWYQQKSGTSPKRWIYDTSKLASGVPGRFSGSGSGNSYSLTISSVEAEDDATYYCQQWSKHPLTYGAGTKLEIK

SEQ ID NO: 21 - protein, 788 aa, synthetic construct
MVSKGEELFTGVVPILVELDGDVNGHKFSVSGEGEGDATYGKLTLKFICTTGKLPVPWPTLVTTLTYGVQCFSRYPDHMKQHDFFKSAMPEGYVQERTIFFKDDGNYKTRAEVKFEGDTLVNRIELKGIDFKEDGNILGHKLEYNYNSHNVYIMADKQKNGIKVNFKIRHNIEDGSVQLADHYQQNTPIGDGPVLLPDNHYLSTQSALSKDPNEKRDHMVLLEFVTAAGITLGMDELYKGSGEGRGSLLTCGDVEENPGPMLLLVTSLLLCELPHPAFLLIPYPYDVPDYAQVQLQQSGPELEKPGASVKISCKASGYSFTGYTMNWVKQSHGKSLEWIGLITPYNGASSYNQKFRGKATLTVDKSSSTAYMDLLSLTSEDSAVYFCARGGYDGRGFDYWGQGTTVTVSSGGGGSGGGGSSGGGSDIELTQSPAIMSASPGEKVTMTCSASSSVSYMHWYQQKSGTSPKRWIYDTSKLASGVPGRFSGSGSGNSYSLTISSVEAEDDATYYCQQWSKHPLTYGAGTKLEIKAAAIEVMYPPPYLDNEKSNGTIIHVKGKHLCPSPLFPGPSKPFWVLVVVGGVLACYSLLVTVAFIIFWVKNRKAKAKGGGGGGDYEPIRKGQRDLYSGLNQRRIRSKRSRLLHSDYMNMTPRRPGPTRKHYQPYAPPRDFAAYRSRVKFSRSADAPAYQQGQNQLYNELNLGRREEYDVLDKRRGRDPEMGGKPRRKNPQEGLYNELQKDKMAEAYSEIGMKGERRRGKGHDGLYQGLSTATKDTYDALHMQALPPR

SEQ ID NO: 22 - protein, 532 aa, synthetic construct
MALPVTALLLPLALLLHAARPYPYDVPDYADIQMTQTTSSLSASLGDRVTISCRASQDISKYLNWYQQKPDGTVKLLIYHTSRLHSGVPSRFSGSGSGTDYSLTISNLEQEDIATYFCQQGNTLPYTFGGGTKLEITGGGGSGGGGSGGGGSEVKLQESGPGLVAPSQSLSVTCTVSGVSLPDYGVSWIRQPPRKGLEWLGVIWGSETTYYNSALKSRLTIIKDNSKSQVFLKMNSLQTDDTAIYYCAKHYYYGGSYAMDYWGQGTSVTVSSASTTTPAPRPPTPAPTIASQPLSLRPEACRPAAGGAVHTRGLDFACDIYIWAPLAGTCGVLLLSLVITLYCKNRKAKAKGGGGGGDYEPIRKGQRDLYSGLNQRRIKRGRKKLLYIFKQPFMRPVQTTQEEDGCSCRFPEEEEGGCELRVKFSRSADAPAYQQGQNQLYNELNLGRREEYDVLDKRRGRDPEMGGKPRRKNPQEGLYNELQKDKMAEAYSEIGMKGERRRGKGHDGLYQGLSTATKDTYDALHMQALPPR

SEQ ID NO: 23 - DNA, 1599 bp, synthetic construct
  source 1..1599: mol_type = other DNA
atggccttaccagtgaccgccttgctcctgccgctggccttgctgctccacgccgccaggccgtacccctacgacgtgcccgactacgccgacatccagatgacacagactacatcctccctgtctgcctctctgggagacagagtcaccatcagttgcagggcaagtcaggacattagtaaatatttaaattggtatcagcagaaaccagatggaactgttaaactcctgatctaccatacatcaagattacactcaggagtcccatcaaggttcagtggcagtgggtctggaacagattattctctcaccattagcaacctggagcaagaagatattgccacttacttttgccaacagggtaatacgcttccgtacacgttcggaggggggaccaagctggagatcacaggtggcggtggctcgggcggtggtgggtcgggtggcggcggatctgaggtgaaactgcaggagtcaggacctggcctggtggcgccctcacagagcctgtccgtcacatgcactgtctcaggggtctcattacccgactatggtgtaagctggattcgccagcctccacgaaagggtctggagtggctgggagtaatatggggtagtgaaaccacatactataattcagctctcaaatccagactgaccatcatcaaggacaactccaagagccaagttttcttaaaaatgaacagtctgcaaactgatgacacagccatttactactgtgccaaacattattactacggtggtagctatgctatggactactggggccaaggaacctcagtcaccgtctcctcagccagtaccaccactcccgcaccccgccctcctactcctgcccctaccattgccagtcaaccgcttagtctgagacctgaggcctgtaggcccgctgctggtggcgctgtgcacacccgaggattggacttcgcttgcgacatctacatctgggcacctctggctgggacctgcggcgtgttgttgttgagcctggtgattacgctgtactgtaagaatagaaaagccaaggctaaaggcggagggggtggcggagactatgagcccatccggaaaggccagcgggacctgtattctggcctgaatcagagacgcatcaaacggggcagaaagaaactcctgtatatattcaaacaaccatttatgagaccagtacaaactactcaagaggaagatggctgtagctgccgatttccagaagaagaagaaggaggatgtgaactgagagtgaagttcagcaggagcgcagacgcccccgcgtaccagcagggccagaaccagctctataacgagctcaatctaggacgaagagaggagtacgatgttttggacaagagacgtggccgggaccctgagatggggggaaagccgagaaggaagaaccctcaggaaggcctgtacaatgaactgcagaaagataagatggcggaggcctacagtgagattgggatgaaaggcgagcgccggaggggcaaggggcacgatggcctttaccagggtctcagtacagccaccaaggacacctacgacgcccttcacatgcaggccctgccccctcgctaa